European Patent Application EP 4 653 454 A1, published November 26, 2025. Title: PROTEIN AND VACCINE AGAINST INFECTION BY SARS-COV-2 OMICRON VARIANT STRAIN AND SUBTYPE THEREOF. Applicant: WestVac Biopharma Co., Ltd. Application CN. The sequence listing filed with the application follows.

SEQUENCE LISTING (42 sequences)

SEQ ID NO: 1 - protein, 324 aa, synthetic construct
VQPTESIVRFPNITNLCPFDEVFNATRFASVYAWNRKRISNCVADYSVLYNFAPFFAFKCYGVSPTKLNDLCFTNVYADSFVIRGNEVSQIAPGQTGNIADYNYKLPDDFTGCVIAWNSNKLDSKVGGNYNYRYRLFRKSNLKPFERDISTEIYQAGNKPCNGVAGVNCYFPLQSYGFRPTYGVGHQPYRVVVLSFELLHAPATVCGPKKSTNLVKNKSVNFNFNGLYENQKLIANQFNSAIGKIQDSLSSTASALGKLQDVVNQNAQALNTLVKQLKNHTSPDVDLGDISGINASVVNIQKEIDRLNEVAKNLNESLIDLQEL

SEQ ID NO: 2 - protein, 324 aa, synthetic construct
VQPTESIVRFPNITNLCPFDEVFNATTFASVYAWNRKRISNCVADYSVLYNFAPFFAFKCYGVSPTKLNDLCFTNVYADSFVIRGNEVSQIAPGQTGNIADYNYKLPDDFTGCVIAWNSNKLDSTVGGNYNYRYRLFRKSKLKPFERDISTEIYQAGNKPCNGVAGVNCYFPLQSYGFRPTYGVGHQPYRVVVLSFELLHAPATVCGPKKSTNLVKNKSVNFNFNGLYENQKLIANQFNSAIGKIQDSLSSTASALGKLQDVVNQNAQALNTLVKQLKNHTSPDVDLGDISGINASVVNIQKEIDRLNEVAKNLNESLIDLQEL

SEQ ID NO: 3 - protein, 324 aa, synthetic construct
VQPTESIVRFPNITNLCPFHEVFNATTFASVYAWNRKRISNCVADYSVIYNFAPFFAFKCYGVSPTKLNDLCFTNVYADSFVIRGNEVSQIAPGQTGNIADYNYKLPDDFTGCVIAWNSNKLDSKPSGNYNYLYRLFRKSKLKPFERDISTEIYQAGNKPCNGVAGPNCYSPLQSYGFRPTYGVGHQPYRVVVLSFELLHAPATVCGPKKSTNLVKNKSVNFNFNGLYENQKLIANQFNSAIGKIQDSLSSTASALGKLQDVVNQNAQALNTLVKQLKNHTSPDVDLGDISGINASVVNIQKEIDRLNEVAKNLNESLIDLQEL

SEQ ID NO: 4 - protein, 1253 aa, synthetic construct
VNLITRTQSYTNSFTRGVYYPDKVFRSSVLHSTQDLFLPFFSNVTWFHAISGTNGTKRFDNPVLPFNDGVYFASTEKSNIIRGWIFGTTLDSKTQSLLIVNNATNVVIKVCEFQFCNDPFLDVYYHKNNKSWMESEFRVYSSANNCTFEYVSQPFLMDLEGKQGNFKNLREFVFKNIDGYFKIYSKHTPINLGRDLPQGFSALEPLVDLPIGINITRFQTLLALHRSYLTPGDSSSGWTAGAAAYYVGYLQPRTFLLKYNENGTITDAVDCALDPLSETKCTLKSFTVEKGIYQTSNFRVQPTESIVRFPNITNLCPFDEVFNATRFASVYAWNRKRISNCVADYSVLYNFAPFFAFKCYGVSPTKLNDLCFTNVYADSFVIRGNEVSQIAPGQTGNIADYNYKLPDDFTGCVIAWNSNKLDSKVGGNYNYRYRLFRKSNLKPFERDISTEIYQAGNKPCNGVAGVNCYFPLQSYGFRPTYGVGHQPYRVVVLSFELLHAPATVCGPKKSTNLVKNKCVNFNFNGLTGTGVLTESNKKFLPFQQFGRDIADTTDAVRDPQTLEILDITPCSFGGVSVITPGTNTSNQVAVLYQGVNCTEVPVAIHADQLTPTWRVYSTGSNVFQTRAGCLIGAEYVNNSYECDIPIGAGICASYQTQTKSHRRARSVASQSIIAYTMSLGAENSVAYSNNSIAIPTNFTISVTTEILPVSMTKTSVDCTMYICGDSTECSNLLLQYGSFCTQLKRALTGIAVEQDKNTQEVFAQVKQIYKTPPIKYFGGFNFSQILPDPSKPSKRSFIEDLLFNKVTLADAGFIKQYGDCLGDIAARDLICAQKFNGLTVLPPLLTDEMIAQYTSALLAGTITSGWTFGAGAALQIPFAMQMAYRFNGIGVTQNVLYENQKLIANQFNSAIGKIQDSLSSTASALGKLQDVVNHNAQALNTLVKQLSSKFGAISSVLNDILSRLDKVEAEVQIDRLITGRLQSLQTYVTQQLIRAAEIRASANLAATKMSECVLGQSKRVDFCGKGYHLMSFPQSAPHGVVFLHVTYVPAQEKNFTTAPAICHDGKAHFPREGVFVSNGTHWFVTQRNFYEPQIITTDNTFVSGNCDVVIGIVNNTVYDPLQPELDSFKEELDKYFKNHTSPDVDLGDISGINASVVNIQKEIDRLNEVAKNLNESLIDLQELGKYEQYIKWPWYIWLGFIAGLIAIVMVTIMLCCMTSCCSCLKGCCSCGSCCKFDEDDSEPVLKGVKLHYT

SEQ ID NO: 5 - protein, 1253 aa, synthetic construct
VNLITRTQSYTNSFTRGVYYPDKVFRSSVLHSTQDLFLPFFSNVTWFHAISGTNGTKRFDNPVLPFNDGVYFASTEKSNIIRGWIFGTTLDSKTQSLLIVNNATNVVIKVCEFQFCNDPFLDVYYHKNNKSWMESEFRVYSSANNCTFEYVSQPFLMDLEGKQGNFKNLREFVFKNIDGYFKIYSKHTPINLGRDLPQGFSALEPLVDLPIGINITRFQTLLALHRSYLTPGDSSSGWTAGAAAYYVGYLQPRTFLLKYNENGTITDAVDCALDPLSETKCTLKSFTVEKGIYQTSNFRVQPTESIVRFPNITNLCPFDEVFNATTFASVYAWNRKRISNCVADYSVLYNFAPFFAFKCYGVSPTKLNDLCFTNVYADSFVIRGNEVSQIAPGQTGNIADYNYKLPDDFTGCVIAWNSNKLDSTVGGNYNYRYRLFRKSKLKPFERDISTEIYQAGNKPCNGVAGVNCYFPLQSYGFRPTYGVGHQPYRVVVLSFELLHAPATVCGPKKSTNLVKNKCVNFNFNGLTGTGVLTESNKKFLPFQQFGRDIADTTDAVRDPQTLEILDITPCSFGGVSVITPGTNTSNQVAVLYQGVNCTEVPVAIHADQLTPTWRVYSTGSNVFQTRAGCLIGAEYVNNSYECDIPIGAGICASYQTQTKSHRRARSVASQSIIAYTMSLGAENSVAYSNNSIAIPTNFTISVTTEILPVSMTKTSVDCTMYICGDSTECSNLLLQYGSFCTQLKRALTGIAVEQDKNTQEVFAQVKQIYKTPPIKYFGGFNFSQILPDPSKPSKRSFIEDLLFNKVTLADAGFIKQYGDCLGDIAARDLICAQKFNGLTVLPPLLTDEMIAQYTSALLAGTITSGWTFGAGAALQIPFAMQMAYRFNGIGVTQNVLYENQKLIANQFNSAIGKIQDSLSSTASALGKLQDVVNHNAQALNTLVKQLSSKFGAISSVLNDILSRLDKVEAEVQIDRLITGRLQSLQTYVTQQLIRAAEIRASANLAATKMSECVLGQSKRVDFCGKGYHLMSFPQSAPHGVVFLHVTYVPAQEKNFTTAPAICHDGKAHFPREGVFVSNGTHWFVTQRNFYEPQIITTDNTFVSGNCDVVIGIVNNTVYDPLQPELDSFKEELDKYFKNHTSPDVDLGDISGINASVVNIQKEIDRLNEVAKNLNESLIDLQELGKYEQYIKWPWYIWLGFIAGLIAIVMVTIMLCCMTSCCSCLKGCCSCGSCCKFDEDDSEPVLKGVKLHYT

SEQ ID NO: 6 - protein, 1254 aa, synthetic construct
VNLITRTQSYTNSFTRGVYYPDKVFRSSVLHSTQDLFLPFFSNVTWFHAIHVSGTNGTKRFDNPALPFNDGVYFASTEKSNIIRGWIFGTTLDSKTQSLLIVNNATNVVIKVCEFQFCNDPFLDVYQKNNKSWMESEFRVYSSANNCTFEYVSQPFLMDLEGKEGNFKNLREFVFKNIDGYFKIYSKHTPINLERDLPQGFSALEPLVDLPIGINITRFQTLLALHRSYLTPVDSSSGWTAGAAAYYVGYLQPRTFLLKYNENGTITDAVDCALDPLSETKCTLKSFTVEKGIYQTSNFRVQPTESIVRFPNITNLCPFHEVFNATTFASVYAWNRKRISNCVADYSVIYNFAPFFAFKCYGVSPTKLNDLCFTNVYADSFVIRGNEVSQIAPGQTGNIADYNYKLPDDFTGCVIAWNSNKLDSKPSGNYNYLYRLFRKSKLKPFERDISTEIYQAGNKPCNGVAGPNCYSPLQSYGFRPTYGVGHQPYRVVVLSFELLHAPATVCGPKKSTNLVKNKCVNFNFNGLTGTGVLTESNKKFLPFQQFGRDIADTTDAVRDPQTLEILDITPCSFGGVSVITPGTNTSNQVAVLYQGVNCTEVPVAIHADQLTPTWRVYSTGSNVFQTRAGCLIGAEYVNNSYECDIPIGAGICASYQTQTKSHRRARSVASQSIIAYTMSLGAENSVAYSNNSIAIPTNFTISVTTEILPVSMTKTSVDCTMYICGDSTECSNLLLQYGSFCTQLKRALTGIAVEQDKNTQEVFAQVKQIYKTPPIKYFGGFNFSQILPDPSKPSKRSFIEDLLFNKVTLADAGFIKQYGDCLGDIAARDLICAQKFNGLTVLPPLLTDEMIAQYTSALLAGTITSGWTFGAGAALQIPFAMQMAYRFNGIGVTQNVLYENQKLIANQFNSAIGKIQDSLSSTASALGKLQDVVNHNAQALNTLVKQLSSKFGAISSVLNDILSRLDKVEAEVQIDRLITGRLQSLQTYVTQQLIRAAEIRASANLAATKMSECVLGQSKRVDFCGKGYHLMSFPQSAPHGVVFLHVTYVPAQEKNFTTAPAICHDGKAHFPREGVFVSNGTHWFVTQRNFYEPQIITTDNTFVSGNCDVVIGIVNNTVYDPLQPELDSFKEELDKYFKNHTSPDVDLGDISGINASVVNIQKEIDRLNEVAKNLNESLIDLQELGKYEQYIKWPWYIWLGFIAGLIAIVMVTIMLCCMTSCCSCLKGCCSCGSCCKFDEDDSEPVLKGVKLHYT

SEQ ID NO: 7 - protein, 324 aa, synthetic construct
VQPTESIVRFPNITNLCPFDEVFNATRFASVYAWNRKRISNCVADYSVLYNSASFSAFKCYGVSPTKLNDLCFTNVYADSFVIRGNEVSQIAPGQTGNIADYNYKLPDDFTGCVIAWNSNKLDSKVGGNYNYRYRLFRKSNLKPFERDISTEIYQAGNKPCNGVAGVNCYFPLQSYGFRPTYGVGHQPYRVVVLSFELLHAPATVCGPKKSTNLVKNKSVNFNFNGLYENQKLIANQFNSAIGKIQDSLSSTASALGKLQDVVNQNAQALNTLVKQLKNHTSPDVDLGDISGINASVVNIQKEIDRLNEVAKNLNESLIDLQEL

SEQ ID NO: 8 - protein, 324 aa, synthetic construct
VQPTESIVRFPNITNLCPFDEVFNATTFASVYAWNRKRISNCVADYSVLYNSASFSAFKCYGVSPTKLNDLCFTNVYADSFVIRGNEVSQIAPGQTGNIADYNYKLPDDFTGCVIAWNSNKLDSTVGGNYNYRYRLFRKSKLKPFERDISTEIYQAGNKPCNGVAGVNCYFPLQSYGFRPTYGVGHQPYRVVVLSFELLHAPATVCGPKKSTNLVKNKSVNFNFNGLYENQKLIANQFNSAIGKIQDSLSSTASALGKLQDVVNQNAQALNTLVKQLKNHTSPDVDLGDISGINASVVNIQKEIDRLNEVAKNLNESLIDLQEL

SEQ ID NO: 9 - protein, 324 aa, synthetic construct
VQPTESIVRFPNITNLCPFHEVFNATTFASVYAWNRKRISNCVADYSVIYNSASFSAFKCYGVSPTKLNDLCFTNVYADSFVIRGNEVSQIAPGQTGNIADYNYKLPDDFTGCVIAWNSNKLDSKPSGNYNYLYRLFRKSKLKPFERDISTEIYQAGNKPCNGVAGPNCYSPLQSYGFRPTYGVGHQPYRVVVLSFELLHAPATVCGPKKSTNLVKNKSVNFNFNGLYENQKLIANQFNSAIGKIQDSLSSTASALGKLQDVVNQNAQALNTLVKQLKNHTSPDVDLGDISGINASVVNIQKEIDRLNEVAKNLNESLIDLQEL

SEQ ID NO: 10 - protein, 1253 aa, synthetic construct
VNLITRTQSYTNSFTRGVYYPDKVFRSSVLHSTQDLFLPFFSNVTWFHAISGTNGTKRFDNPVLPFNDGVYFASTEKSNIIRGWIFGTTLDSKTQSLLIVNNATNVVIKVCEFQFCNDPFLDVYYHKNNKSWMESEFRVYSSANNCTFEYVSQPFLMDLEGKQGNFKNLREFVFKNIDGYFKIYSKHTPINLGRDLPQGFSALEPLVDLPIGINITRFQTLLALHRSYLTPGDSSSGWTAGAAAYYVGYLQPRTFLLKYNENGTITDAVDCALDPLSETKCTLKSFTVEKGIYQTSNFRVQPTESIVRFPNITNLCPFDEVFNATRFASVYAWNRKRISNCVADYSVLYNSASFSAFKCYGVSPTKLNDLCFTNVYADSFVIRGNEVSQIAPGQTGNIADYNYKLPDDFTGCVIAWNSNKLDSKVGGNYNYRYRLFRKSNLKPFERDISTEIYQAGNKPCNGVAGVNCYFPLQSYGFRPTYGVGHQPYRVVVLSFELLHAPATVCGPKKSTNLVKNKCVNFNFNGLTGTGVLTESNKKFLPFQQFGRDIADTTDAVRDPQTLEILDITPCSFGGVSVITPGTNTSNQVAVLYQGVNCTEVPVAIHADQLTPTWRVYSTGSNVFQTRAGCLIGAEYVNNSYECDIPIGAGICASYQTQTKSHRRARSVASQSIIAYTMSLGAENSVAYSNNSIAIPTNFTISVTTEILPVSMTKTSVDCTMYICGDSTECSNLLLQYGSFCTQLKRALTGIAVEQDKNTQEVFAQVKQIYKTPPIKYFGGFNFSQILPDPSKPSKRSFIEDLLFNKVTLADAGFIKQYGDCLGDIAARDLICAQKFNGLTVLPPLLTDEMIAQYTSALLAGTITSGWTFGAGAALQIPFAMQMAYRFNGIGVTQNVLYENQKLIANQFNSAIGKIQDSLSSTASALGKLQDVVNHNAQALNTLVKQLSSKFGAISSVLNDILSRLDKVEAEVQIDRLITGRLQSLQTYVTQQLIRAAEIRASANLAATKMSECVLGQSKRVDFCGKGYHLMSFPQSAPHGVVFLHVTYVPAQEKNFTTAPAICHDGKAHFPREGVFVSNGTHWFVTQRNFYEPQIITTDNTFVSGNCDVVIGIVNNTVYDPLQPELDSFKEELDKYFKNHTSPDVDLGDISGINASVVNIQKEIDRLNEVAKNLNESLIDLQELGKYEQYIKWPWYIWLGFIAGLIAIVMVTIMLCCMTSCCSCLKGCCSCGSCCKFDEDDSEPVLKGVKLHYT

SEQ ID NO: 11 - protein, 1253 aa, synthetic construct
VNLITRTQSYTNSFTRGVYYPDKVFRSSVLHSTQDLFLPFFSNVTWFHAISGTNGTKRFDNPVLPFNDGVYFASTEKSNIIRGWIFGTTLDSKTQSLLIVNNATNVVIKVCEFQFCNDPFLDVYYHKNNKSWMESEFRVYSSANNCTFEYVSQPFLMDLEGKQGNFKNLREFVFKNIDGYFKIYSKHTPINLGRDLPQGFSALEPLVDLPIGINITRFQTLLALHRSYLTPGDSSSGWTAGAAAYYVGYLQPRTFLLKYNENGTITDAVDCALDPLSETKCTLKSFTVEKGIYQTSNFRVQPTESIVRFPNITNLCPFDEVFNATTFASVYAWNRKRISNCVADYSVLYNSASFSAFKCYGVSPTKLNDLCFTNVYADSFVIRGNEVSQIAPGQTGNIADYNYKLPDDFTGCVIAWNSNKLDSTVGGNYNYRYRLFRKSKLKPFERDISTEIYQAGNKPCNGVAGVNCYFPLQSYGFRPTYGVGHQPYRVVVLSFELLHAPATVCGPKKSTNLVKNKCVNFNFNGLTGTGVLTESNKKFLPFQQFGRDIADTTDAVRDPQTLEILDITPCSFGGVSVITPGTNTSNQVAVLYQGVNCTEVPVAIHADQLTPTWRVYSTGSNVFQTRAGCLIGAEYVNNSYECDIPIGAGICASYQTQTKSHRRARSVASQSIIAYTMSLGAENSVAYSNNSIAIPTNFTISVTTEILPVSMTKTSVDCTMYICGDSTECSNLLLQYGSFCTQLKRALTGIAVEQDKNTQEVFAQVKQIYKTPPIKYFGGFNFSQILPDPSKPSKRSFIEDLLFNKVTLADAGFIKQYGDCLGDIAARDLICAQKFNGLTVLPPLLTDEMIAQYTSALLAGTITSGWTFGAGAALQIPFAMQMAYRFNGIGVTQNVLYENQKLIANQFNSAIGKIQDSLSSTASALGKLQDVVNHNAQALNTLVKQLSSKFGAISSVLNDILSRLDKVEAEVQIDRLITGRLQSLQTYVTQQLIRAAEIRASANLAATKMSECVLGQSKRVDFCGKGYHLMSFPQSAPHGVVFLHVTYVPAQEKNFTTAPAICHDGKAHFPREGVFVSNGTHWFVTQRNFYEPQIITTDNTFVSGNCDVVIGIVNNTVYDPLQPELDSFKEELDKYFKNHTSPDVDLGDISGINASVVNIQKEIDRLNEVAKNLNESLIDLQELGKYEQYIKWPWYIWLGFIAGLIAIVMVTIMLCCMTSCCSCLKGCCSCGSCCKFDEDDSEPVLKGVKLHYT

SEQ ID NO: 12 - protein, 1254 aa, synthetic construct
VNLITRTQSYTNSFTRGVYYPDKVFRSSVLHSTQDLFLPFFSNVTWFHAIHVSGTNGTKRFDNPALPFNDGVYFASTEKSNIIRGWIFGTTLDSKTQSLLIVNNATNVVIKVCEFQFCNDPFLDVYQKNNKSWMESEFRVYSSANNCTFEYVSQPFLMDLEGKEGNFKNLREFVFKNIDGYFKIYSKHTPINLERDLPQGFSALEPLVDLPIGINITRFQTLLALHRSYLTPVDSSSGWTAGAAAYYVGYLQPRTFLLKYNENGTITDAVDCALDPLSETKCTLKSFTVEKGIYQTSNFRVQPTESIVRFPNITNLCPFHEVFNATTFASVYAWNRKRISNCVADYSVIYNSASFSAFKCYGVSPTKLNDLCFTNVYADSFVIRGNEVSQIAPGQTGNIADYNYKLPDDFTGCVIAWNSNKLDSKPSGNYNYLYRLFRKSKLKPFERDISTEIYQAGNKPCNGVAGPNCYSPLQSYGFRPTYGVGHQPYRVVVLSFELLHAPATVCGPKKSTNLVKNKCVNFNFNGLTGTGVLTESNKKFLPFQQFGRDIADTTDAVRDPQTLEILDITPCSFGGVSVITPGTNTSNQVAVLYQGVNCTEVPVAIHADQLTPTWRVYSTGSNVFQTRAGCLIGAEYVNNSYECDIPIGAGICASYQTQTKSHRRARSVASQSIIAYTMSLGAENSVAYSNNSIAIPTNFTISVTTEILPVSMTKTSVDCTMYICGDSTECSNLLLQYGSFCTQLKRALTGIAVEQDKNTQEVFAQVKQIYKTPPIKYFGGFNFSQILPDPSKPSKRSFIEDLLFNKVTLADAGFIKQYGDCLGDIAARDLICAQKFNGLTVLPPLLTDEMIAQYTSALLAGTITSGWTFGAGAALQIPFAMQMAYRFNGIGVTQNVLYENQKLIANQFNSAIGKIQDSLSSTASALGKLQDVVNHNAQALNTLVKQLSSKFGAISSVLNDILSRLDKVEAEVQIDRLITGRLQSLQTYVTQQLIRAAEIRASANLAATKMSECVLGQSKRVDFCGKGYHLMSFPQSAPHGVVFLHVTYVPAQEKNFTTAPAICHDGKAHFPREGVFVSNGTHWFVTQRNFYEPQIITTDNTFVSGNCDVVIGIVNNTVYDPLQPELDSFKEELDKYFKNHTSPDVDLGDISGINASVVNIQKEIDRLNEVAKNLNESLIDLQELGKYEQYIKWPWYIWLGFIAGLIAIVMVTIMLCCMTSCCSCLKGCCSCGSCCKFDEDDSEPVLKGVKLHYT

SEQ ID NO: 13 - protein, 492 aa, synthetic construct
MLLVNQSHQGFNKEHTSKMVSAIVLYVLLAAAAHSAFAADSIHIKDSDDLKNRLAEAGDKLVVIDFMATWCGPCKMIGPKLDEMANEMSDSIVVLKVDVDECEDIATEYNINSMPTFVFVKNSKKIEEFSGANVDKLRNTIIKLKLAGSGSGHMHHHHHHSSGDDDDKVQPTESIVRFPNITNLCPFDEVFNATRFASVYAWNRKRISNCVADYSVLYNFAPFFAFKCYGVSPTKLNDLCFTNVYADSFVIRGNEVSQIAPGQTGNIADYNYKLPDDFTGCVIAWNSNKLDSKVGGNYNYRYRLFRKSNLKPFERDISTEIYQAGNKPCNGVAGVNCYFPLQSYGFRPTYGVGHQPYRVVVLSFELLHAPATVCGPKKSTNLVKNKSVNFNFNGLYENQKLIANQFNSAIGKIQDSLSSTASALGKLQDVVNQNAQALNTLVKQLKNHTSPDVDLGDISGINASVVNIQKEIDRLNEVAKNLNESLIDLQEL

SEQ ID NO: 14 - protein, 492 aa, synthetic construct
MLLVNQSHQGFNKEHTSKMVSAIVLYVLLAAAAHSAFAADSIHIKDSDDLKNRLAEAGDKLVVIDFMATWCGPCKMIGPKLDEMANEMSDSIVVLKVDVDECEDIATEYNINSMPTFVFVKNSKKIEEFSGANVDKLRNTIIKLKLAGSGSGHMHHHHHHSSGDDDDKVQPTESIVRFPNITNLCPFDEVFNATTFASVYAWNRKRISNCVADYSVLYNFAPFFAFKCYGVSPTKLNDLCFTNVYADSFVIRGNEVSQIAPGQTGNIADYNYKLPDDFTGCVIAWNSNKLDSTVGGNYNYRYRLFRKSKLKPFERDISTEIYQAGNKPCNGVAGVNCYFPLQSYGFRPTYGVGHQPYRVVVLSFELLHAPATVCGPKKSTNLVKNKSVNFNFNGLYENQKLIANQFNSAIGKIQDSLSSTASALGKLQDVVNQNAQALNTLVKQLKNHTSPDVDLGDISGINASVVNIQKEIDRLNEVAKNLNESLIDLQEL

SEQ ID NO: 15 - protein, 492 aa, synthetic construct
MLLVNQSHQGFNKEHTSKMVSAIVLYVLLAAAAHSAFAADSIHIKDSDDLKNRLAEAGDKLVVIDFMATWCGPCKMIGPKLDEMANEMSDSIVVLKVDVDECEDIATEYNINSMPTFVFVKNSKKIEEFSGANVDKLRNTIIKLKLAGSGSGHMHHHHHHSSGDDDDKVQPTESIVRFPNITNLCPFHEVFNATTFASVYAWNRKRISNCVADYSVIYNFAPFFAFKCYGVSPTKLNDLCFTNVYADSFVIRGNEVSQIAPGQTGNIADYNYKLPDDFTGCVIAWNSNKLDSKPSGNYNYLYRLFRKSKLKPFERDISTEIYQAGNKPCNGVAGPNCYSPLQSYGFRPTYGVGHQPYRVVVLSFELLHAPATVCGPKKSTNLVKNKSVNFNFNGLYENQKLIANQFNSAIGKIQDSLSSTASALGKLQDVVNQNAQALNTLVKQLKNHTSPDVDLGDISGINASVVNIQKEIDRLNEVAKNLNESLIDLQEL

SEQ ID NO: 16 - protein, 1268 aa, synthetic construct
MFVFLVLLPLVSSQCVNLITRTQSYTNSFTRGVYYPDKVFRSSVLHSTQDLFLPFFSNVTWFHAISGTNGTKRFDNPVLPFNDGVYFASTEKSNIIRGWIFGTTLDSKTQSLLIVNNATNVVIKVCEFQFCNDPFLDVYYHKNNKSWMESEFRVYSSANNCTFEYVSQPFLMDLEGKQGNFKNLREFVFKNIDGYFKIYSKHTPINLGRDLPQGFSALEPLVDLPIGINITRFQTLLALHRSYLTPGDSSSGWTAGAAAYYVGYLQPRTFLLKYNENGTITDAVDCALDPLSETKCTLKSFTVEKGIYQTSNFRVQPTESIVRFPNITNLCPFDEVFNATRFASVYAWNRKRISNCVADYSVLYNFAPFFAFKCYGVSPTKLNDLCFTNVYADSFVIRGNEVSQIAPGQTGNIADYNYKLPDDFTGCVIAWNSNKLDSKVGGNYNYRYRLFRKSNLKPFERDISTEIYQAGNKPCNGVAGVNCYFPLQSYGFRPTYGVGHQPYRVVVLSFELLHAPATVCGPKKSTNLVKNKCVNFNFNGLTGTGVLTESNKKFLPFQQFGRDIADTTDAVRDPQTLEILDITPCSFGGVSVITPGTNTSNQVAVLYQGVNCTEVPVAIHADQLTPTWRVYSTGSNVFQTRAGCLIGAEYVNNSYECDIPIGAGICASYQTQTKSHRRARSVASQSIIAYTMSLGAENSVAYSNNSIAIPTNFTISVTTEILPVSMTKTSVDCTMYICGDSTECSNLLLQYGSFCTQLKRALTGIAVEQDKNTQEVFAQVKQIYKTPPIKYFGGFNFSQILPDPSKPSKRSFIEDLLFNKVTLADAGFIKQYGDCLGDIAARDLICAQKFNGLTVLPPLLTDEMIAQYTSALLAGTITSGWTFGAGAALQIPFAMQMAYRFNGIGVTQNVLYENQKLIANQFNSAIGKIQDSLSSTASALGKLQDVVNHNAQALNTLVKQLSSKFGAISSVLNDILSRLDKVEAEVQIDRLITGRLQSLQTYVTQQLIRAAEIRASANLAATKMSECVLGQSKRVDFCGKGYHLMSFPQSAPHGVVFLHVTYVPAQEKNFTTAPAICHDGKAHFPREGVFVSNGTHWFVTQRNFYEPQIITTDNTFVSGNCDVVIGIVNNTVYDPLQPELDSFKEELDKYFKNHTSPDVDLGDISGINASVVNIQKEIDRLNEVAKNLNESLIDLQELGKYEQYIKWPWYIWLGFIAGLIAIVMVTIMLCCMTSCCSCLKGCCSCGSCCKFDEDDSEPVLKGVKLHYT

SEQ ID NO: 17 - protein, 1268 aa, synthetic construct
MFVFLVLLPLVSSQCVNLITRTQSYTNSFTRGVYYPDKVFRSSVLHSTQDLFLPFFSNVTWFHAISGTNGTKRFDNPVLPFNDGVYFASTEKSNIIRGWIFGTTLDSKTQSLLIVNNATNVVIKVCEFQFCNDPFLDVYYHKNNKSWMESEFRVYSSANNCTFEYVSQPFLMDLEGKQGNFKNLREFVFKNIDGYFKIYSKHTPINLGRDLPQGFSALEPLVDLPIGINITRFQTLLALHRSYLTPGDSSSGWTAGAAAYYVGYLQPRTFLLKYNENGTITDAVDCALDPLSETKCTLKSFTVEKGIYQTSNFRVQPTESIVRFPNITNLCPFDEVFNATTFASVYAWNRKRISNCVADYSVLYNFAPFFAFKCYGVSPTKLNDLCFTNVYADSFVIRGNEVSQIAPGQTGNIADYNYKLPDDFTGCVIAWNSNKLDSTVGGNYNYRYRLFRKSKLKPFERDISTEIYQAGNKPCNGVAGVNCYFPLQSYGFRPTYGVGHQPYRVVVLSFELLHAPATVCGPKKSTNLVKNKCVNFNFNGLTGTGVLTESNKKFLPFQQFGRDIADTTDAVRDPQTLEILDITPCSFGGVSVITPGTNTSNQVAVLYQGVNCTEVPVAIHADQLTPTWRVYSTGSNVFQTRAGCLIGAEYVNNSYECDIPIGAGICASYQTQTKSHRRARSVASQSIIAYTMSLGAENSVAYSNNSIAIPTNFTISVTTEILPVSMTKTSVDCTMYICGDSTECSNLLLQYGSFCTQLKRALTGIAVEQDKNTQEVFAQVKQIYKTPPIKYFGGFNFSQILPDPSKPSKRSFIEDLLFNKVTLADAGFIKQYGDCLGDIAARDLICAQKFNGLTVLPPLLTDEMIAQYTSALLAGTITSGWTFGAGAALQIPFAMQMAYRFNGIGVTQNVLYENQKLIANQFNSAIGKIQDSLSSTASALGKLQDVVNHNAQALNTLVKQLSSKFGAISSVLNDILSRLDKVEAEVQIDRLITGRLQSLQTYVTQQLIRAAEIRASANLAATKMSECVLGQSKRVDFCGKGYHLMSFPQSAPHGVVFLHVTYVPAQEKNFTTAPAICHDGKAHFPREGVFVSNGTHWFVTQRNFYEPQIITTDNTFVSGNCDVVIGIVNNTVYDPLQPELDSFKEELDKYFKNHTSPDVDLGDISGINASVVNIQKEIDRLNEVAKNLNESLIDLQELGKYEQYIKWPWYIWLGFIAGLIAIVMVTIMLCCMTSCCSCLKGCCSCGSCCKFDEDDSEPVLKGVKLHYT

SEQ ID NO: 18 - protein, 1269 aa, synthetic construct
MFVFLVLLPLVSSQCVNLITRTQSYTNSFTRGVYYPDKVFRSSVLHSTQDLFLPFFSNVTWFHAIHVSGTNGTKRFDNPALPFNDGVYFASTEKSNIIRGWIFGTTLDSKTQSLLIVNNATNVVIKVCEFQFCNDPFLDVYQKNNKSWMESEFRVYSSANNCTFEYVSQPFLMDLEGKEGNFKNLREFVFKNIDGYFKIYSKHTPINLERDLPQGFSALEPLVDLPIGINITRFQTLLALHRSYLTPVDSSSGWTAGAAAYYVGYLQPRTFLLKYNENGTITDAVDCALDPLSETKCTLKSFTVEKGIYQTSNFRVQPTESIVRFPNITNLCPFHEVFNATTFASVYAWNRKRISNCVADYSVIYNFAPFFAFKCYGVSPTKLNDLCFTNVYADSFVIRGNEVSQIAPGQTGNIADYNYKLPDDFTGCVIAWNSNKLDSKPSGNYNYLYRLFRKSKLKPFERDISTEIYQAGNKPCNGVAGPNCYSPLQSYGFRPTYGVGHQPYRVVVLSFELLHAPATVCGPKKSTNLVKNKCVNFNFNGLTGTGVLTESNKKFLPFQQFGRDIADTTDAVRDPQTLEILDITPCSFGGVSVITPGTNTSNQVAVLYQGVNCTEVPVAIHADQLTPTWRVYSTGSNVFQTRAGCLIGAEYVNNSYECDIPIGAGICASYQTQTKSHRRARSVASQSIIAYTMSLGAENSVAYSNNSIAIPTNFTISVTTEILPVSMTKTSVDCTMYICGDSTECSNLLLQYGSFCTQLKRALTGIAVEQDKNTQEVFAQVKQIYKTPPIKYFGGFNFSQILPDPSKPSKRSFIEDLLFNKVTLADAGFIKQYGDCLGDIAARDLICAQKFNGLTVLPPLLTDEMIAQYTSALLAGTITSGWTFGAGAALQIPFAMQMAYRFNGIGVTQNVLYENQKLIANQFNSAIGKIQDSLSSTASALGKLQDVVNHNAQALNTLVKQLSSKFGAISSVLNDILSRLDKVEAEVQIDRLITGRLQSLQTYVTQQLIRAAEIRASANLAATKMSECVLGQSKRVDFCGKGYHLMSFPQSAPHGVVFLHVTYVPAQEKNFTTAPAICHDGKAHFPREGVFVSNGTHWFVTQRNFYEPQIITTDNTFVSGNCDVVIGIVNNTVYDPLQPELDSFKEELDKYFKNHTSPDVDLGDISGINASVVNIQKEIDRLNEVAKNLNESLIDLQELGKYEQYIKWPWYIWLGFIAGLIAIVMVTIMLCCMTSCCSCLKGCCSCGSCCKFDEDDSEPVLKGVKLHYT

SEQ ID NO: 19 - protein, 492 aa, synthetic construct
MLLVNQSHQGFNKEHTSKMVSAIVLYVLLAAAAHSAFAADSIHIKDSDDLKNRLAEAGDKLVVIDFMATWCGPCKMIGPKLDEMANEMSDSIVVLKVDVDECEDIATEYNINSMPTFVFVKNSKKIEEFSGANVDKLRNTIIKLKLAGSGSGHMHHHHHHSSGDDDDKVQPTESIVRFPNITNLCPFDEVFNATRFASVYAWNRKRISNCVADYSVLYNSASFSAFKCYGVSPTKLNDLCFTNVYADSFVIRGNEVSQIAPGQTGNIADYNYKLPDDFTGCVIAWNSNKLDSKVGGNYNYRYRLFRKSNLKPFERDISTEIYQAGNKPCNGVAGVNCYFPLQSYGFRPTYGVGHQPYRVVVLSFELLHAPATVCGPKKSTNLVKNKSVNFNFNGLYENQKLIANQFNSAIGKIQDSLSSTASALGKLQDVVNQNAQALNTLVKQLKNHTSPDVDLGDISGINASVVNIQKEIDRLNEVAKNLNESLIDLQEL

SEQ ID NO: 20 - protein, 492 aa, synthetic construct
MLLVNQSHQGFNKEHTSKMVSAIVLYVLLAAAAHSAFAADSIHIKDSDDLKNRLAEAGDKLVVIDFMATWCGPCKMIGPKLDEMANEMSDSIVVLKVDVDECEDIATEYNINSMPTFVFVKNSKKIEEFSGANVDKLRNTIIKLKLAGSGSGHMHHHHHHSSGDDDDKVQPTESIVRFPNITNLCPFDEVFNATTFASVYAWNRKRISNCVADYSVLYNSASFSAFKCYGVSPTKLNDLCFTNVYADSFVIRGNEVSQIAPGQTGNIADYNYKLPDDFTGCVIAWNSNKLDSTVGGNYNYRYRLFRKSKLKPFERDISTEIYQAGNKPCNGVAGVNCYFPLQSYGFRPTYGVGHQPYRVVVLSFELLHAPATVCGPKKSTNLVKNKSVNFNFNGLYENQKLIANQFNSAIGKIQDSLSSTASALGKLQDVVNQNAQALNTLVKQLKNHTSPDVDLGDISGINASVVNIQKEIDRLNEVAKNLNESLIDLQEL

SEQ ID NO: 21 - protein, 492 aa, synthetic construct
MLLVNQSHQGFNKEHTSKMVSAIVLYVLLAAAAHSAFAADSIHIKDSDDLKNRLAEAGDKLVVIDFMATWCGPCKMIGPKLDEMANEMSDSIVVLKVDVDECEDIATEYNINSMPTFVFVKNSKKIEEFSGANVDKLRNTIIKLKLAGSGSGHMHHHHHHSSGDDDDKVQPTESIVRFPNITNLCPFHEVFNATTFASVYAWNRKRISNCVADYSVIYNSASFSAFKCYGVSPTKLNDLCFTNVYADSFVIRGNEVSQIAPGQTGNIADYNYKLPDDFTGCVIAWNSNKLDSKPSGNYNYLYRLFRKSKLKPFERDISTEIYQAGNKPCNGVAGPNCYSPLQSYGFRPTYGVGHQPYRVVVLSFELLHAPATVCGPKKSTNLVKNKSVNFNFNGLYENQKLIANQFNSAIGKIQDSLSSTASALGKLQDVVNQNAQALNTLVKQLKNHTSPDVDLGDISGINASVVNIQKEIDRLNEVAKNLNESLIDLQEL

SEQ ID NO: 22 - protein, 1268 aa, synthetic construct
MFVFLVLLPLVSSQCVNLITRTQSYTNSFTRGVYYPDKVFRSSVLHSTQDLFLPFFSNVTWFHAISGTNGTKRFDNPVLPFNDGVYFASTEKSNIIRGWIFGTTLDSKTQSLLIVNNATNVVIKVCEFQFCNDPFLDVYYHKNNKSWMESEFRVYSSANNCTFEYVSQPFLMDLEGKQGNFKNLREFVFKNIDGYFKIYSKHTPINLGRDLPQGFSALEPLVDLPIGINITRFQTLLALHRSYLTPGDSSSGWTAGAAAYYVGYLQPRTFLLKYNENGTITDAVDCALDPLSETKCTLKSFTVEKGIYQTSNFRVQPTESIVRFPNITNLCPFDEVFNATRFASVYAWNRKRISNCVADYSVLYNSASFSAFKCYGVSPTKLNDLCFTNVYADSFVIRGNEVSQIAPGQTGNIADYNYKLPDDFTGCVIAWNSNKLDSKVGGNYNYRYRLFRKSNLKPFERDISTEIYQAGNKPCNGVAGVNCYFPLQSYGFRPTYGVGHQPYRVVVLSFELLHAPATVCGPKKSTNLVKNKCVNFNFNGLTGTGVLTESNKKFLPFQQFGRDIADTTDAVRDPQTLEILDITPCSFGGVSVITPGTNTSNQVAVLYQGVNCTEVPVAIHADQLTPTWRVYSTGSNVFQTRAGCLIGAEYVNNSYECDIPIGAGICASYQTQTKSHRRARSVASQSIIAYTMSLGAENSVAYSNNSIAIPTNFTISVTTEILPVSMTKTSVDCTMYICGDSTECSNLLLQYGSFCTQLKRALTGIAVEQDKNTQEVFAQVKQIYKTPPIKYFGGFNFSQILPDPSKPSKRSFIEDLLFNKVTLADAGFIKQYGDCLGDIAARDLICAQKFNGLTVLPPLLTDEMIAQYTSALLAGTITSGWTFGAGAALQIPFAMQMAYRFNGIGVTQNVLYENQKLIANQFNSAIGKIQDSLSSTASALGKLQDVVNHNAQALNTLVKQLSSKFGAISSVLNDILSRLDKVEAEVQIDRLITGRLQSLQTYVTQQLIRAAEIRASANLAATKMSECVLGQSKRVDFCGKGYHLMSFPQSAPHGVVFLHVTYVPAQEKNFTTAPAICHDGKAHFPREGVFVSNGTHWFVTQRNFYEPQIITTDNTFVSGNCDVVIGIVNNTVYDPLQPELDSFKEELDKYFKNHTSPDVDLGDISGINASVVNIQKEIDRLNEVAKNLNESLIDLQELGKYEQYIKWPWYIWLGFIAGLIAIVMVTIMLCCMTSCCSCLKGCCSCGSCCKFDEDDSEPVLKGVKLHYT

SEQ ID NO: 23 - protein, 1268 aa, synthetic construct
MFVFLVLLPLVSSQCVNLITRTQSYTNSFTRGVYYPDKVFRSSVLHSTQDLFLPFFSNVTWFHAISGTNGTKRFDNPVLPFNDGVYFASTEKSNIIRGWIFGTTLDSKTQSLLIVNNATNVVIKVCEFQFCNDPFLDVYYHKNNKSWMESEFRVYSSANNCTFEYVSQPFLMDLEGKQGNFKNLREFVFKNIDGYFKIYSKHTPINLGRDLPQGFSALEPLVDLPIGINITRFQTLLALHRSYLTPGDSSSGWTAGAAAYYVGYLQPRTFLLKYNENGTITDAVDCALDPLSETKCTLKSFTVEKGIYQTSNFRVQPTESIVRFPNITNLCPFDEVFNATTFASVYAWNRKRISNCVADYSVLYNSASFSAFKCYGVSPTKLNDLCFTNVYADSFVIRGNEVSQIAPGQTGNIADYNYKLPDDFTGCVIAWNSNKLDSTVGGNYNYRYRLFRKSKLKPFERDISTEIYQAGNKPCNGVAGVNCYFPLQSYGFRPTYGVGHQPYRVVVLSFELLHAPATVCGPKKSTNLVKNKCVNFNFNGLTGTGVLTESNKKFLPFQQFGRDIADTTDAVRDPQTLEILDITPCSFGGVSVITPGTNTSNQVAVLYQGVNCTEVPVAIHADQLTPTWRVYSTGSNVFQTRAGCLIGAEYVNNSYECDIPIGAGICASYQTQTKSHRRARSVASQSIIAYTMSLGAENSVAYSNNSIAIPTNFTISVTTEILPVSMTKTSVDCTMYICGDSTECSNLLLQYGSFCTQLKRALTGIAVEQDKNTQEVFAQVKQIYKTPPIKYFGGFNFSQILPDPSKPSKRSFIEDLLFNKVTLADAGFIKQYGDCLGDIAARDLICAQKFNGLTVLPPLLTDEMIAQYTSALLAGTITSGWTFGAGAALQIPFAMQMAYRFNGIGVTQNVLYENQKLIANQFNSAIGKIQDSLSSTASALGKLQDVVNHNAQALNTLVKQLSSKFGAISSVLNDILSRLDKVEAEVQIDRLITGRLQSLQTYVTQQLIRAAEIRASANLAATKMSECVLGQSKRVDFCGKGYHLMSFPQSAPHGVVFLHVTYVPAQEKNFTTAPAICHDGKAHFPREGVFVSNGTHWFVTQRNFYEPQIITTDNTFVSGNCDVVIGIVNNTVYDPLQPELDSFKEELDKYFKNHTSPDVDLGDISGINASVVNIQKEIDRLNEVAKNLNESLIDLQELGKYEQYIKWPWYIWLGFIAGLIAIVMVTIMLCCMTSCCSCLKGCCSCGSCCKFDEDDSEPVLKGVKLHYT

SEQ ID NO: 24 - protein, 1269 aa, synthetic construct
MFVFLVLLPLVSSQCVNLITRTQSYTNSFTRGVYYPDKVFRSSVLHSTQDLFLPFFSNVTWFHAIHVSGTNGTKRFDNPALPFNDGVYFASTEKSNIIRGWIFGTTLDSKTQSLLIVNNATNVVIKVCEFQFCNDPFLDVYQKNNKSWMESEFRVYSSANNCTFEYVSQPFLMDLEGKEGNFKNLREFVFKNIDGYFKIYSKHTPINLERDLPQGFSALEPLVDLPIGINITRFQTLLALHRSYLTPVDSSSGWTAGAAAYYVGYLQPRTFLLKYNENGTITDAVDCALDPLSETKCTLKSFTVEKGIYQTSNFRVQPTESIVRFPNITNLCPFHEVFNATTFASVYAWNRKRISNCVADYSVIYNSASFSAFKCYGVSPTKLNDLCFTNVYADSFVIRGNEVSQIAPGQTGNIADYNYKLPDDFTGCVIAWNSNKLDSKPSGNYNYLYRLFRKSKLKPFERDISTEIYQAGNKPCNGVAGPNCYSPLQSYGFRPTYGVGHQPYRVVVLSFELLHAPATVCGPKKSTNLVKNKCVNFNFNGLTGTGVLTESNKKFLPFQQFGRDIADTTDAVRDPQTLEILDITPCSFGGVSVITPGTNTSNQVAVLYQGVNCTEVPVAIHADQLTPTWRVYSTGSNVFQTRAGCLIGAEYVNNSYECDIPIGAGICASYQTQTKSHRRARSVASQSIIAYTMSLGAENSVAYSNNSIAIPTNFTISVTTEILPVSMTKTSVDCTMYICGDSTECSNLLLQYGSFCTQLKRALTGIAVEQDKNTQEVFAQVKQIYKTPPIKYFGGFNFSQILPDPSKPSKRSFIEDLLFNKVTLADAGFIKQYGDCLGDIAARDLICAQKFNGLTVLPPLLTDEMIAQYTSALLAGTITSGWTFGAGAALQIPFAMQMAYRFNGIGVTQNVLYENQKLIANQFNSAIGKIQDSLSSTASALGKLQDVVNHNAQALNTLVKQLSSKFGAISSVLNDILSRLDKVEAEVQIDRLITGRLQSLQTYVTQQLIRAAEIRASANLAATKMSECVLGQSKRVDFCGKGYHLMSFPQSAPHGVVFLHVTYVPAQEKNFTTAPAICHDGKAHFPREGVFVSNGTHWFVTQRNFYEPQIITTDNTFVSGNCDVVIGIVNNTVYDPLQPELDSFKEELDKYFKNHTSPDVDLGDISGINASVVNIQKEIDRLNEVAKNLNESLIDLQELGKYEQYIKWPWYIWLGFIAGLIAIVMVTIMLCCMTSCCSCLKGCCSCGSCCKFDEDDSEPVLKGVKLHYT

SEQ ID NO: 25 - DNA, 1479 bp, synthetic construct
  source 1..1479: mol_type = other DNA
atgctgctggtgaaccagagccaccagggtttcaacaaggaacacactagcaagatggtgtctgctatcgtcctctacgtgctgctcgccgccgctgctcactcagctttcgccgctgactctatccacatcaaggactccgacgacctcaagaaccgtttggccgaagccggcgacaagctggtcgttatcgacttcatggctacctggtgtggcccttgcaagatgatcggacctaagctggacgaaatggctaacgagatgagcgacagcatcgtcgttctgaaggtggacgtcgacgaatgtgaggacatcgccactgagtacaacatcaacagcatgcctaccttcgttttcgtgaagaactctaagaagatcgaggagttctctggtgccaacgtggacaagctccgtaacaccatcatcaagctcaagctggccggcagcggtagcggtcacatgcaccaccaccaccaccattcaagcggcgacgacgacgacaaggtgcagccaaccgaatcaatcgtccgcttcccaaacatcactaacctgtgcccattcgacgaggtgttcaacgccacccgtttcgcctctgtctacgcttggaaccgcaagcgcatctccaactgtgtcgccgactacagcgtgctgtacaacttcgctcctttcttcgcattcaagtgttacggagtgtcccctaccaagctcaacgatttgtgcttcacaaacgtgtacgctgacagcttcgtgatccgtggtaacgaggtttctcaaatcgcccctggtcagacaggtaacatcgctgactacaactacaagctcccagacgacttcactggctgtgttatcgcttggaactcaaacaagctggactctaaggtgggtggtaactacaactaccggtaccgtctgttccgcaagagcaacctcaagccattcgaacgtgacatcagcacagagatctaccaagccggtaacaagccctgcaacggcgttgccggagtcaactgctacttccccctccagtcctacggattccgcccaacctacggcgtgggtcaccagccataccgcgtggttgtgctgagcttcgaactgctgcacgcccccgctaccgtgtgtggccctaagaagagcactaacctcgttaagaacaagtccgtgaacttcaacttcaacggtctctacgaaaaccagaagctgatcgctaaccagttcaactccgccatcggcaagatccaggactccctgtcctccacagcttccgctctgggcaagctgcaggacgttgtgaaccaaaacgctcaggccctgaacacactggtgaagcaactgaagaaccacaccagccccgacgttgacctgggtgacatcagcggtatcaacgctagcgtggtgaacatccagaaggagatcgacaggctgaacgaagtggctaagaacttgaacgagagcctcatcgacctgcaggaactgtaa

SEQ ID NO: 26 - DNA, 1479 bp, synthetic construct
  source 1..1479: mol_type = other DNA
atgctgctggtgaaccagagccaccagggtttcaacaaggaacacactagcaagatggtgtctgctatcgtcctctacgtgctgctcgccgccgctgctcactcagctttcgccgctgactctatccacatcaaggactccgacgacctcaagaaccgtttggccgaagccggcgacaagctggtcgttatcgacttcatggctacctggtgtggcccttgcaagatgatcggacctaagctggacgaaatggctaacgagatgagcgacagcatcgtcgttctgaaggtggacgtcgacgaatgtgaggacatcgccactgagtacaacatcaacagcatgcctaccttcgttttcgtgaagaactctaagaagatcgaggagttctctggtgccaacgtggacaagctccgtaacaccatcatcaagctcaagctggccggcagcggtagcggtcacatgcaccaccaccaccaccattcaagcggcgacgacgacgacaaggtgcagccaaccgaatcaatcgtccgcttcccaaacatcactaacctgtgcccattcgacgaggtgttcaacgccaccactttcgcctctgtctacgcttggaaccgcaagcgcatctccaactgtgtcgccgactacagcgtgctgtacaacttcgctcctttcttcgcattcaagtgttacggagtgtcccctaccaagctcaacgatttgtgcttcacaaacgtgtacgctgacagcttcgtgatccgtggtaacgaggtttctcaaatcgcccctggtcagacaggtaacatcgctgactacaactacaagctcccagacgacttcactggctgtgttatcgcttggaactcaaacaagctggactctactgtgggtggtaactacaactaccggtaccgtctgttccgcaagagcaagctcaagccattcgaacgtgacatcagcacagagatctaccaagccggtaacaagccctgcaacggcgttgccggagtcaactgctacttccccctccagtcctacggattccgcccaacctacggcgtgggtcaccagccataccgcgtggttgtgctgagcttcgaactgctgcacgcccccgctaccgtgtgtggccctaagaagagcactaacctcgttaagaacaagtccgtgaacttcaacttcaacggtctctacgaaaaccagaagctgatcgctaaccagttcaactccgccatcggcaagatccaggactccctgtcctccacagcttccgctctgggcaagctgcaggacgttgtgaaccaaaacgctcaggccctgaacacactggtgaagcaactgaagaaccacaccagccccgacgttgacctgggtgacatcagcggtatcaacgctagcgtggtgaacatccagaaggagatcgacaggctgaacgaagtggctaagaacttgaacgagagcctcatcgacctgcaggaactgtaa

SEQ ID NO: 27 - DNA, 1479 bp, synthetic construct
  source 1..1479: mol_type = other DNA
atgctgctggtgaaccagagccaccagggtttcaacaaggaacacactagcaagatggtgtctgctatcgtcctctacgtgctgctcgccgccgctgctcactcagctttcgccgctgactctatccacatcaaggactccgacgacctcaagaaccgtttggccgaagccggcgacaagctggtcgttatcgacttcatggctacctggtgtggcccttgcaagatgatcggacctaagctggacgaaatggctaacgagatgagcgacagcatcgtcgttctgaaggtggacgtcgacgaatgtgaggacatcgccactgagtacaacatcaacagcatgcctaccttcgttttcgtgaagaactctaagaagatcgaggagttctctggtgccaacgtggacaagctccgtaacaccatcatcaagctcaagctggccggcagcggtagcggtcacatgcaccaccaccaccaccattcaagcggcgacgacgacgacaaggtgcagccaaccgaatcaatcgtccgcttcccaaacatcactaacctgtgcccattccacgaggtgttcaacgccaccactttcgcctctgtctacgcttggaaccgcaagcgcatctccaactgtgtcgccgactacagcgtgatatacaacttcgctcctttcttcgcattcaagtgttacggagtgtcccctaccaagctcaacgatttgtgcttcacaaacgtgtacgctgacagcttcgtgatccgtggtaacgaggtttctcaaatcgcccctggtcagacaggtaacatcgctgactacaactacaagctcccagacgacttcactggctgtgttatcgcttggaactcaaacaagctggactctaagccgtctggtaactacaactacctctaccgtctgttccgcaagagcaagctcaagccattcgaacgtgacatcagcacagagatctaccaagccggtaacaagccctgcaacggcgttgccggacctaactgctactctcccctccagtcctacggattccgcccaacctacggcgtgggtcaccagccataccgcgtggttgtgctgagcttcgaactgctgcacgcccccgctaccgtgtgtggccctaagaagagcactaacctcgttaagaacaagtccgtgaacttcaacttcaacggtctctacgaaaaccagaagctgatcgctaaccagttcaactccgccatcggcaagatccaggactccctgtcctccacagcttccgctctgggcaagctgcaggacgttgtgaaccaaaacgctcaggccctgaacacactggtgaagcaactgaagaaccacaccagccccgacgttgacctgggtgacatcagcggtatcaacgctagcgtggtgaacatccagaaggagatcgacaggctgaacgaagtggctaagaacttgaacgagagcctcatcgacctgcaggaactgtaa

SEQ ID NO: 28 - DNA, 1479 bp, synthetic construct
  source 1..1479: mol_type = other DNA
atgctgctggtgaaccagagccaccagggtttcaacaaggaacacactagcaagatggtgtctgctatcgtcctctacgtgctgctcgccgccgctgctcactcagctttcgccgctgactctatccacatcaaggactccgacgacctcaagaaccgtttggccgaagccggcgacaagctggtcgttatcgacttcatggctacctggtgtggcccttgcaagatgatcggacctaagctggacgaaatggctaacgagatgagcgacagcatcgtcgttctgaaggtggacgtcgacgaatgtgaggacatcgccactgagtacaacatcaacagcatgcctaccttcgttttcgtgaagaactctaagaagatcgaggagttctctggtgccaacgtggacaagctccgtaacaccatcatcaagctcaagctggccggcagcggtagcggtcacatgcaccaccaccaccaccattcaagcggcgacgacgacgacaaggtgcagccaaccgaatcaatcgtccgcttcccaaacatcactaacctgtgcccattcgacgaggtgttcaacgccacccgtttcgcctctgtctacgcttggaaccgcaagcgcatctccaactgtgtcgccgactacagcgtgctgtacaactcagcttcattctcagcattcaagtgttacggagtgtcccctaccaagctcaacgatttgtgcttcacaaacgtgtacgctgacagcttcgtgatccgtggtaacgaggtttctcaaatcgcccctggtcagacaggtaacatcgctgactacaactacaagctcccagacgacttcactggctgtgttatcgcttggaactcaaacaagctggactctaaggtgggtggtaactacaactaccggtaccgtctgttccgcaagagcaacctcaagccattcgaacgtgacatcagcacagagatctaccaagccggtaacaagccctgcaacggcgttgccggagtcaactgctacttccccctccagtcctacggattccgcccaacctacggcgtgggtcaccagccataccgcgtggttgtgctgagcttcgaactgctgcacgcccccgctaccgtgtgtggccctaagaagagcactaacctcgttaagaacaagtccgtgaacttcaacttcaacggtctctacgaaaaccagaagctgatcgctaaccagttcaactccgccatcggcaagatccaggactccctgtcctccacagcttccgctctgggcaagctgcaggacgttgtgaaccaaaacgctcaggccctgaacacactggtgaagcaactgaagaaccacaccagccccgacgttgacctgggtgacatcagcggtatcaacgctagcgtggtgaacatccagaaggagatcgacaggctgaacgaagtggctaagaacttgaacgagagcctcatcgacctgcaggaactgtaa

SEQ ID NO: 29 - DNA, 1479 bp, synthetic construct
  source 1..1479: mol_type = other DNA
atgctgctggtgaaccagagccaccagggtttcaacaaggaacacactagcaagatggtgtctgctatcgtcctctacgtgctgctcgccgccgctgctcactcagctttcgccgctgactctatccacatcaaggactccgacgacctcaagaaccgtttggccgaagccggcgacaagctggtcgttatcgacttcatggctacctggtgtggcccttgcaagatgatcggacctaagctggacgaaatggctaacgagatgagcgacagcatcgtcgttctgaaggtggacgtcgacgaatgtgaggacatcgccactgagtacaacatcaacagcatgcctaccttcgttttcgtgaagaactctaagaagatcgaggagttctctggtgccaacgtggacaagctccgtaacaccatcatcaagctcaagctggccggcagcggtagcggtcacatgcaccaccaccaccaccattcaagcggcgacgacgacgacaaggtgcagccaaccgaatcaatcgtccgcttcccaaacatcactaacctgtgcccattcgacgaggtgttcaacgccaccactttcgcctctgtctacgcttggaaccgcaagcgcatctccaactgtgtcgccgactacagcgtgctgtacaactccgcttctttctccgcattcaagtgttacggagtgtcccctaccaagctcaacgatttgtgcttcacaaacgtgtacgctgacagcttcgtgatccgtggtaacgaggtttctcaaatcgcccctggtcagacaggtaacatcgctgactacaactacaagctcccagacgacttcactggctgtgttatcgcttggaactcaaacaagctggactctactgtgggtggtaactacaactaccggtaccgtctgttccgcaagagcaagctcaagccattcgaacgtgacatcagcacagagatctaccaagccggtaacaagccctgcaacggcgttgccggagtcaactgctacttccccctccagtcctacggattccgcccaacctacggcgtgggtcaccagccataccgcgtggttgtgctgagcttcgaactgctgcacgcccccgctaccgtgtgtggccctaagaagagcactaacctcgttaagaacaagtccgtgaacttcaacttcaacggtctctacgaaaaccagaagctgatcgctaaccagttcaactccgccatcggcaagatccaggactccctgtcctccacagcttccgctctgggcaagctgcaggacgttgtgaaccaaaacgctcaggccctgaacacactggtgaagcaactgaagaaccacaccagccccgacgttgacctgggtgacatcagcggtatcaacgctagcgtggtgaacatccagaaggagatcgacaggctgaacgaagtggctaagaacttgaacgagagcctcatcgacctgcaggaactgtaa

SEQ ID NO: 30 - DNA, 1479 bp, synthetic construct
  source 1..1479: mol_type = other DNA
atgctgctggtgaaccagagccaccagggtttcaacaaggaacacactagcaagatggtgtctgctatcgtcctctacgtgctgctcgccgccgctgctcactcagctttcgccgctgactctatccacatcaaggactccgacgacctcaagaaccgtttggccgaagccggcgacaagctggtcgttatcgacttcatggctacctggtgtggcccttgcaagatgatcggacctaagctggacgaaatggctaacgagatgagcgacagcatcgtcgttctgaaggtggacgtcgacgaatgtgaggacatcgccactgagtacaacatcaacagcatgcctaccttcgttttcgtgaagaactctaagaagatcgaggagttctctggtgccaacgtggacaagctccgtaacaccatcatcaagctcaagctggccggcagcggtagcggtcacatgcaccaccaccaccaccattcaagcggcgacgacgacgacaaggtgcagccaaccgaatcaatcgtccgcttcccaaacatcactaacctgtgcccattccacgaggtgttcaacgccaccactttcgcctctgtctacgcttggaaccgcaagcgcatctccaactgtgtcgccgactacagcgtgatatacaactccgcttctttctctgcattcaagtgttacggagtgtcccctaccaagctcaacgatttgtgcttcacaaacgtgtacgctgacagcttcgtgatccgtggtaacgaggtttctcaaatcgcccctggtcagacaggtaacatcgctgactacaactacaagctcccagacgacttcactggctgtgttatcgcttggaactcaaacaagctggactctaagccgtctggtaactacaactacctctaccgtctgttccgcaagagcaagctcaagccattcgaacgtgacatcagcacagagatctaccaagccggtaacaagccctgcaacggcgttgccggacctaactgctactctcccctccagtcctacggattccgcccaacctacggcgtgggtcaccagccataccgcgtggttgtgctgagcttcgaactgctgcacgcccccgctaccgtgtgtggccctaagaagagcactaacctcgttaagaacaagtccgtgaacttcaacttcaacggtctctacgaaaaccagaagctgatcgctaaccagttcaactccgccatcggcaagatccaggactccctgtcctccacagcttccgctctgggcaagctgcaggacgttgtgaaccaaaacgctcaggccctgaacacactggtgaagcaactgaagaaccacaccagccccgacgttgacctgggtgacatcagcggtatcaacgctagcgtggtgaacatccagaaggagatcgacaggctgaacgaagtggctaagaacttgaacgagagcctcatcgacctgcaggaactgtaa

SEQ ID NO: 31 - protein, 492 aa, synthetic construct
MLLVNQSHQGFNKEHTSKMVSAIVLYVLLAAAAHSAFAADSIHIKDSDDLKNRLAEAGDKLVVIDFMATWCGPCKMIGPKLDEMANEMSDSIVVLKVDVDECEDIATEYNINSMPTFVFVKNSKKIEEFSGANVDKLRNTIIKLKLAGSGSGHMHHHHHHSSGDDDDKVQPTESIVRFPNITNLCPFGEVFNATRFASVYAWNRKRISNCVADYSVLYNSASFSTFKCYGVSPTKLNDLCFTNVYADSFVIRGDEVRQIAPGQTGKIADYNYKLPDDFTGCVIAWNSNNLDSKVGGNYNYRYRLFRKSNLKPFERDISTEIYQAGSKPCNGVEGFNCYFPLQSYGFQPTNGVGYQPYRVVVLSFELLHAPATVCGPKKSTNLVKNKSVNFNFNGLYENQKLIANQFNSAIGKIQDSLSSTASALGKLQDVVNQNAQALNTLVKQLKNHTSPDVDLGDISGINASVVNIQKEIDRLNEVAKNLNESLIDLQEL

SEQ ID NO: 32 - DNA, 1479 bp, synthetic construct
  source 1..1479: mol_type = other DNA
atgctactagtaaatcagtcacaccaaggcttcaataaggaacacacaagcaagatggtgagcgctatcgtgctgtacgtcctgctggccgctgctgctcacagcgctttcgctgctgactccatccacatcaaggacagcgacgacctgaagaaccgtctggccgaggccggtgacaagctggtcgtcatcgacttcatggccacttggtgcggtccttgcaagatgatcggccctaagctggacgagatggctaacgagatgtccgacagcatcgtggtcctgaaggtggacgtcgacgagtgcgaggacatcgccaccgaatacaacatcaacagcatgcccaccttcgtgttcgtgaagaacagcaagaagatcgaggaattttccggcgctaacgtcgacaagctgcgtaacaccatcatcaagctgaagctggccggctccggctccggccacatgcatcaccaccaccaccattcctccggtgacgacgacgacaaggtgcagccaaccgaatctatcgtcagattcccaaacatcactaacctgtgccctttcggagaggtgttcaacgctaccaggttcgccagcgtctacgcttggaaccgcaagcgtatcagcaactgcgtcgccgactactctgtgctgtacaactccgctagcttctctactttcaagtgctacggcgtgtcacctaccaagctgaacgacctgtgcttcactaacgtctacgccgactccttcgtgatccgcggagacgaagtccgtcagatcgctcctggacagaccggaaagatcgctgactacaactacaagctgccagacgacttcactggctgcgtgatcgcttggaactcaaacaacctggactccaaggtcggtggcaactacaactaccggtacaggctgttcagaaagtcaaacctgaagcctttcgagcgcgacatctcaaccgaaatctaccaggctggttccaagccctgcaacggtgtggagggcttcaactgctacttccccctgcagtcctacggtttccagccaaccaacggagtcggttaccagccttaccgtgtggtcgtgctgagcttcgaactgctccacgctcctgctactgtgtgcggtcccaagaagtctactaacctggtcaaaaacaaaagcgtcaacttcaacttcaacggtctgtacgagaaccagaagctgatcgctaaccagttcaacagcgccatcggcaagatccaggactcactgtcatccactgcctccgctctgggaaagctgcaggacgtcgtgaaccagaacgcccaggctctgaacaccctggtcaagcagctgaagaaccacacctctcctgacgtcgacctgggcgacatcagcggaatcaacgcttctgtcgtgaacatccagaaggagatcgaccgcctgaacgaagtggccaagaacctgaacgaatccctgattgacctccaagaactctaa

SEQ ID NO: 33 - protein, 1271 aa, synthetic construct
MFVFLVLLPLVSSQCVNLRTRTQLPPAYTNSFTRGVYYPDKVFRSSVLHSTQDLFLPFFSNVTWFHAIHVSGTNGTKRFDNPVLPFNDGVYFASTEKSNIIRGWIFGTTLDSKTQSLLIVNNATNVVIKVCEFQFCNDPFLDVYYHKNNKSWMESGVYSSANNCTFEYVSQPFLMDLEGKQGNFKNLREFVFKNIDGYFKIYSKHTPINLVRDLPQGFSALEPLVDLPIGINITRFQTLLALHRSYLTPGDSSSGWTAGAAAYYVGYLQPRTFLLKYNENGTITDAVDCALDPLSETKCTLKSFTVEKGIYQTSNFRVQPTESIVRFPNITNLCPFGEVFNATRFASVYAWNRKRISNCVADYSVLYNSASFSTFKCYGVSPTKLNDLCFTNVYADSFVIRGDEVRQIAPGQTGKIADYNYKLPDDFTGCVIAWNSNNLDSKVGGNYNYRYRLFRKSNLKPFERDISTEIYQAGSKPCNGVEGFNCYFPLQSYGFQPTNGVGYQPYRVVVLSFELLHAPATVCGPKKSTNLVKNKCVNFNFNGLTGTGVLTESNKKFLPFQQFGRDIADTTDAVRDPQTLEILDITPCSFGGVSVITPGTNTSNQVAVLYQGVNCTEVPVAIHADQLTPTWRVYSTGSNVFQTRAGCLIGAEHVNNSYECDIPIGAGICASYQTQTNSRRRARSVASQSIIAYTMSLGAENSVAYSNNSIAIPTNFTISVTTEILPVSMTKTSVDCTMYICGDSTECSNLLLQYGSFCTQLNRALTGIAVEQDKNTQEVFAQVKQIYKTPPIKDFGGFNFSQILPDPSKPSKRSFIEDLLFNKVTLADAGFIKQYGDCLGDIAARDLICAQKFNGLTVLPPLLTDEMIAQYTSALLAGTITSGWTFGAGAALQIPFAMQMAYRFNGIGVTQNVLYENQKLIANQFNSAIGKIQDSLSSTASALGKLQNVVNQNAQALNTLVKQLSSNFGAISSVLNDILSRLDKVEAEVQIDRLITGRLQSLQTYVTQQLIRAAEIRASANLAATKMSECVLGQSKRVDFCGKGYHLMSFPQSAPHGVVFLHVTYVPAQEKNFTTAPAICHDGKAHFPREGVFVSNGTHWFVTQRNFYEPQIITTDNTFVSGNCDVVIGIVNNTVYDPLQPELDSFKEELDKYFKNHTSPDVDLGDISGINASVVNIQKEIDRLNEVAKNLNESLIDLQELGKYEQYIKWPWYIWLGFIAGLIAIVMVTIMLCCMTSCCSCLKGCCSCGSCCKFDEDDSEPVLKGVKLHYT

SEQ ID NO: 34 - protein, 1267 aa, synthetic construct
MFVFLVLLPLVSSQCVNLTTRTQLPPAYTNSFTRGVYYPDKVFRSSVLHSTQDLFLPFFSNVTWFHVISGTNGTKRFDNPVLPFNDGVYFASIEKSNIIRGWIFGTTLDSKTQSLLIVNNATNVVIKVCEFQFCNDPFLDHKNNKSWMESEFRVYSSANNCTFEYVSQPFLMDLEGKQGNFKNLREFVFKNIDGYFKIYSKHTPIIVRDLPQGFSALEPLVDLPIGINITRFQTLLALHRSYLTPGDSSSGWTAGAAAYYVGYLQPRTFLLKYNENGTITDAVDCALDPLSETKCTLKSFTVEKGIYQTSNFRVQPTESIVRFPNITNLCPFDEVFNATRFASVYAWNRKRISNCVADYSVLYNLAPFFTFKCYGVSPTKLNDLCFTNVYADSFVIRGDEVRQIAPGQTGNIADYNYKLPDDFTGCVIAWNSNKLDSKVSGNYNYLYRLFRKSNLKPFERDISTEIYQAGNKPCNGVAGFNCYFPLRSYSFRPTYGVGHQPYRVVVLSFELLHAPATVCGPKKSTNLVKNKCVNFNFNGLKGTGVLTESNKKFLPFQQFGRDIADTTDAVRDPQTLEILDITPCSFGGVSVITPGTNTSNQVAVLYQGVNCTEVPVAIHADQLTPTWRVYSTGSNVFQTRAGCLIGAEYVNNSYECDIPIGAGICASYQTQTKSHRRARSVASQSIIAYTMSLGAENSVAYSNNSIAIPTNFTISVTTEILPVSMTKTSVDCTMYICGDSTECSNLLLQYGSFCTQLKRALTGIAVEQDKNTQEVFAQVKQIYKTPPIKYFGGFNFSQILPDPSKPSKRSFIEDLLFNKVTLADAGFIKQYGDCLGDIAARDLICAQKFKGLTVLPPLLTDEMIAQYTSALLAGTITSGWTFGAGAALQIPFAMQMAYRFNGIGVTQNVLYENQKLIANQFNSAIGKIQDSLSSTASALGKLQDVVNHNAQALNTLVKQLSSKFGAISSVLNDIFSRLDKVEAEVQIDRLITGRLQSLQTYVTQQLIRAAEIRASANLAATKMSECVLGQSKRVDFCGKGYHLMSFPQSAPHGVVFLHVTYVPAQEKNFTTAPAICHDGKAHFPREGVFVSNGTHWFVTQRNFYEPQIITTDNTFVSGNCDVVIGIVNNTVYDPLQPELDSFKEELDKYFKNHTSPDVDLGDISGINASVVNIQKEIDRLNEVAKNLNESLIDLQELGKYEQYIKWPWYIWLGFIAGLIAIVMVTIMLCCMTSCCSCLKGCCSCGSCCKFDEDDSEPVLKGVKLHYT

SEQ ID NO: 35 - protein, 1267 aa, synthetic construct
MFVFLVLLPLVSSQCVNLTTRTQLPPAYTNSFTRGVYYPDKVFRSSVLHSTQDLFLPFFSNVTWFHVISGTNGTKRFDNPVLPFNDGVYFASIEKSNIIRGWIFGTTLDSKTQSLLIVNNATNVVIKVCEFQFCNDPFLDHKNNKSWMESEFRVYSSANNCTFEYVSQPFLMDLEGKQGNFKNLREFVFKNIDGYFKIYSKHTPIIVRDLPQGFSALEPLVDLPIGINITRFQTLLALHRSYLTPGDSSSGWTAGAAAYYVGYLQPRTFLLKYNENGTITDAVDCALDPLSETKCTLKSFTVEKGIYQTSNFRVQPTESIVRFPNITNLCPFDEVFNATRFASVYAWNRKRISNCVADYSVLYNSASFSTFKCYGVSPTKLNDLCFTNVYADSFVIRGDEVRQIAPGQTGNIADYNYKLPDDFTGCVIAWNSNKLDSKVSGNYNYLYRLFRKSNLKPFERDISTEIYQAGNKPCNGVAGFNCYFPLRSYSFRPTYGVGHQPYRVVVLSFELLHAPATVCGPKKSTNLVKNKCVNFNFNGLKGTGVLTESNKKFLPFQQFGRDIADTTDAVRDPQTLEILDITPCSFGGVSVITPGTNTSNQVAVLYQGVNCTEVPVAIHADQLTPTWRVYSTGSNVFQTRAGCLIGAEYVNNSYECDIPIGAGICASYQTQTKSHRRARSVASQSIIAYTMSLGAENSVAYSNNSIAIPTNFTISVTTEILPVSMTKTSVDCTMYICGDSTECSNLLLQYGSFCTQLKRALTGIAVEQDKNTQEVFAQVKQIYKTPPIKYFGGFNFSQILPDPSKPSKRSFIEDLLFNKVTLADAGFIKQYGDCLGDIAARDLICAQKFKGLTVLPPLLTDEMIAQYTSALLAGTITSGWTFGAGAALQIPFAMQMAYRFNGIGVTQNVLYENQKLIANQFNSAIGKIQDSLSSTASALGKLQDVVNHNAQALNTLVKQLSSKFGAISSVLNDIFSRLDKVEAEVQIDRLITGRLQSLQTYVTQQLIRAAEIRASANLAATKMSECVLGQSKRVDFCGKGYHLMSFPQSAPHGVVFLHVTYVPAQEKNFTTAPAICHDGKAHFPREGVFVSNGTHWFVTQRNFYEPQIITTDNTFVSGNCDVVIGIVNNTVYDPLQPELDSFKEELDKYFKNHTSPDVDLGDISGINASVVNIQKEIDRLNEVAKNLNESLIDLQELGKYEQYIKWPWYIWLGFIAGLIAIVMVTIMLCCMTSCCSCLKGCCSCGSCCKFDEDDSEPVLKGVKLHYT

SEQ ID NO: 36 - protein, 324 aa, synthetic construct
VQPTESIVRFPNITNLCPFGEVFNATRFASVYAWNRKRISNCVADYSVLYNSASFSTFKCYGVSPTKLNDLCFTNVYADSFVIRGDEVRQIAPGQTGKIADYNYKLPDDFTGCVIAWNSNNLDSKVGGNYNYRYRLFRKSNLKPFERDISTEIYQAGSKPCNGVEGFNCYFPLQSYGFQPTNGVGYQPYRVVVLSFELLHAPATVCGPKKSTNLVKNKSVNFNFNGLYENQKLIANQFNSAIGKIQDSLSSTASALGKLQDVVNQNAQALNTLVKQLKNHTSPDVDLGDISGINASVVNIQKEIDRLNEVAKNLNESLIDLQEL

SEQ ID NO: 37 - protein, 492 aa, synthetic construct
MLLVNQSHQGFNKEHTSKMVSAIVLYVLLAAAAHSAFAADSIHIKDSDDLKNRLAEAGDKLVVIDFMATWCGPCKMIGPKLDEMANEMSDSIVVLKVDVDECEDIATEYNINSMPTFVFVKNSKKIEEFSGANVDKLRNTIIKLKLAGSGSGHMHHHHHHSSGDDDDKVQPTESIVRFPNITNLCPFDEVFNATRFASVYAWNRKRISNCVADYSVLYNLAPFFTFKCYGVSPTKLNDLCFTNVYADSFVIRGDEVRQIAPGQTGNIADYNYKLPDDFTGCVIAWNSNKLDSKVSGNYNYLYRLFRKSNLKPFERDISTEIYQAGNKPCNGVAGFNCYFPLRSYSFRPTYGVGHQPYRVVVLSFELLHAPATVCGPKKSTNLVKNKSVNFNFNGLYENQKLIANQFNSAIGKIQDSLSSTASALGKLQDVVNQNAQALNTLVKQLKNHTSPDVDLGDISGINASVVNIQKEIDRLNEVAKNLNESLIDLQEL

SEQ ID NO: 38 - DNA, 1479 bp, synthetic construct
  source 1..1479: mol_type = other DNA
atgctgctggtgaaccagagccaccagggtttcaacaaggaacacactagcaagatggtgtctgctatcgtcctctacgtgctgctcgccgccgctgctcactcagctttcgccgctgactctatccacatcaaggactccgacgacctcaagaaccgtttggccgaagccggcgacaagctggtcgttatcgacttcatggctacctggtgtggcccttgcaagatgatcggacctaagctggacgaaatggctaacgagatgagcgacagcatcgtcgttctgaaggtggacgtcgacgaatgtgaggacatcgccactgagtacaacatcaacagcatgcctaccttcgttttcgtgaagaactctaagaagatcgaggagttctctggtgccaacgtggacaagctccgtaacaccatcatcaagctcaagctggccggcagcggtagcggtcacatgcaccaccaccaccaccattcaagcggcgacgacgacgacaaggtgcagccaaccgaatcaatcgtccgcttcccaaacatcactaacctgtgcccattcgacgaggtgttcaacgccacccgtttcgcctctgtctacgcttggaaccgcaagcgcatctccaactgtgtcgccgactacagcgtgctgtacaaccttgctcctttcttcaccttcaagtgttacggagtgtcccctaccaagctcaacgatttgtgcttcacaaacgtgtacgctgacagcttcgtgatccgtggtgacgaggttcgccaaatcgcccctggtcagacaggtaacatcgctgactacaactacaagctcccagacgacttcactggctgtgttatcgcttggaactcaaacaagctggactctaaggtgtctggtaactacaactacctctaccgtctgttccgcaagagcaacctcaagccattcgaacgtgacatcagcacagagatctaccaagccggtaacaagccctgcaacggcgttgccggattcaactgctacttccccctccgttcctactcattccgcccaacctacggcgtgggtcaccagccataccgcgtggttgtgctgagcttcgaactgctgcacgcccccgctaccgtgtgtggccctaagaagagcactaacctcgttaagaacaagtccgtgaacttcaacttcaacggtctctacgaaaaccagaagctgatcgctaaccagttcaactccgccatcggcaagatccaggactccctgtcctccacagcttccgctctgggcaagctgcaggacgttgtgaaccaaaacgctcaggccctgaacacactggtgaagcaactgaagaaccacaccagccccgacgttgacctgggtgacatcagcggtatcaacgctagcgtggtgaacatccagaaggagatcgacaggctgaacgaagtggctaagaacttgaacgagagcctcatcgacctgcaggaactgtaa

SEQ ID NO: 39 - protein, 324 aa, synthetic construct
VQPTESIVRFPNITNLCPFDEVFNATRFASVYAWNRKRISNCVADYSVLYNLAPFFTFKCYGVSPTKLNDLCFTNVYADSFVIRGDEVRQIAPGQTGNIADYNYKLPDDFTGCVIAWNSNKLDSKVSGNYNYLYRLFRKSNLKPFERDISTEIYQAGNKPCNGVAGFNCYFPLRSYSFRPTYGVGHQPYRVVVLSFELLHAPATVCGPKKSTNLVKNKSVNFNFNGLYENQKLIANQFNSAIGKIQDSLSSTASALGKLQDVVNQNAQALNTLVKQLKNHTSPDVDLGDISGINASVVNIQKEIDRLNEVAKNLNESLIDLQEL

SEQ ID NO: 40 - DNA, 20 bp, synthetic construct
  source 1..20: mol_type = other DNA
gaccccaaaatcagcgaaat

SEQ ID NO: 41 - DNA, 25 bp, synthetic construct
  source 1..25: mol_type = other DNA
tctggttactgcccagttgaatctg

SEQ ID NO: 42 - DNA, 25 bp, synthetic construct
  source 1..25: mol_type = other DNA
acgccgcattacgtttggtgggacc